European Patent Application EP 4 382 537 A1, published June 12, 2024. Title: 항 CD154 항체 및 이의 용도. Applicant: SEOUL NATIONAL UNIVERSITY R&DB FOUNDATION. The sequence listing filed with the application follows.

SEQUENCE LISTING (15 sequences)

SEQ ID NO: 1 - protein, 10 aa, synthetic construct
GFTFSSYGMQ

SEQ ID NO: 2 - protein, 17 aa, synthetic construct
AIDDDGSSTNYGAAVKG

SEQ ID NO: 3 - protein, 16 aa, synthetic construct
DGIIYYWNADAGYIDA

SEQ ID NO: 4 - protein, 8 aa, synthetic construct
SGGSGSYG

SEQ ID NO: 5 - protein, 7 aa, synthetic construct
WDDERPS

SEQ ID NO: 6 - protein, 11 aa, synthetic construct
GGYDDSSYAGI

SEQ ID NO: 7 - protein, 103 aa, synthetic construct
LTQPSSVSANPGETVKITCSGGSGSYGWYQQKSPGSAPVTLIYWDDERPSDIPSRFSGSKSGSTATLTITGVQAEDEAVYFCGGYDDSSYAGIFGAGTTLTVL

SEQ ID NO: 8 - protein, 127 aa, synthetic construct
AVTLDESGGGLHTPGGALSLVCKASGFTFSSYGMQWVRQAPGKGLEFVAAIDDDGSSTNYGAAVKGRATISRDNGQSTVRLQLNNLRAEDTGTYYCAKDGIIYYWNADAGYIDAWGHGTEVIVSSTS

SEQ ID NO: 9 - protein, 103 aa, synthetic construct
LTQPSSVSANPGETVKITCSGGSGSYGWYQQKSPGSAPVTVIYWDDERPSDIPDRFSGSKSGSTASLTITGVQAEDEAVYYCGGYDDSSYAGIFGAGTTLTVL

SEQ ID NO: 10 - protein, 127 aa, synthetic construct
AVTLVESGGGLHTPGGALRLSCAASGFTFSSYGMQWVRQAPGKGLEFVAAIDDDGSSTNYGAAVKGRATISRDNGQSTLYLQMNSLRAEDTGTYYCAKDGIIYYWNADAGYIDAWGQGTEVIVSSTS

SEQ ID NO: 11 - protein, 103 aa, synthetic construct
LTQPSSVSANPGETVKITCSGGSGSYGWYQQRSPGSAPTTVIYWDDERPSDIPDRFSGSKSGSTASLTITGVQAEDEADYYCGGYDDSSYAGIFGGGTKLTVL

SEQ ID NO: 12 - protein, 127 aa, synthetic construct
AVHLVESGGGLVTPGGALRLSCAASGFTFSSYGMQWVRQAPGKGLEFVAAIDDDGSSTNYGAAVKGRFTISRDNGQSTLYLQMNSLRAEDTAVYYCAKDGIIYYWNADAGYIDAWGQGTLVTVSSTS

SEQ ID NO: 13 - protein, 103 aa, synthetic construct
LTQPSSVSVSPGQTARITCSGGSGSYGWYQQRSPGSAPTTVIYWDDERPSDIPDRFSGSKSGSTASLTISGVQAEDEADYYCGGYDDSSYAGIFGGGTKLTVL

SEQ ID NO: 14 - protein, 127 aa, synthetic construct; identical to SEQ ID NO: 12

SEQ ID NO: 15 - protein, 18 aa, synthetic construct
GQSSRSSGGGGSSGGGGS